European Patent Application EP 4 212 542 A1, published July 19, 2023. Title: BISPECIFIC FUSION POLYPEPTIDE COMPOUND. Applicant: SHAANXI MICOT TECHNOLOGY CO., LTD. The sequence listing filed with the application follows.

SEQUENCE LISTING (28 sequences)

SEQ ID NO: 1 - protein, 7 aa, Artificial Sequence
  MOD_RES (1)..(1): Cys is acetylated
  MOD_RES (6)..(6): Xaa is D-Ala
  MOD_RES (7)..(7): Arg is amidated
CARRRXR

SEQ ID NO: 2 - protein, 5 aa, Artificial Sequence
YCFGG

SEQ ID NO: 3 - protein, 5 aa, Artificial Sequence
  MOD_RES (1)..(1): Xaa is D-Tyr
  MOD_RES (3)..(3): Xaa is D-Phe
XCXGG

SEQ ID NO: 4 - protein, 5 aa, Artificial Sequence
  MOD_RES (1)..(1): Xaa is D-Tyr
  MOD_RES (2)..(2): Xaa is D-Cys
  MOD_RES (3)..(3): Xaa is D-Phe
XXXGG

SEQ ID NO: 5 - protein, 6 aa, Artificial Sequence
  MOD_RES (1)..(1): Xaa is D-Tyr
  UNSURE (2)..(2): Xaa is Aib
  MOD_RES (3)..(3): Xaa is D-Phe
XXXGGC

SEQ ID NO: 6 - protein, 6 aa, Artificial Sequence
  MOD_RES (1)..(1): Xaa is D-Tyr
  MOD_RES (2)..(2): Xaa is D-Arg
  MOD_RES (3)..(3): Xaa is D-Phe
XXXGGC

SEQ ID NO: 7 - protein, 7 aa, Artificial Sequence
  MOD_RES (1)..(1): Xaa is D-Cys acetylated
  MOD_RES (2)..(2): Xaa is D-Ala
  MOD_RES (3)..(3): Xaa is D-Arg
  MOD_RES (4)..(4): Xaa is D-Arg
  MOD_RES (5)..(5): Xaa is D-Arg
  MOD_RES (6)..(6): Xaa is D-Ala
  MOD_RES (7)..(7): Xaa is D-Arg amidated
  BINDING (1)..(1): Xaa is Cys linked to Cys in SEQ ID NO: 2 via a disulfide bond
XXXXXXX

SEQ ID NO: 8 - protein, 7 aa, Artificial Sequence
  MOD_RES (1)..(1): Xaa is D-Cys acetylated
  MOD_RES (2)..(2): Xaa is D-Ala
  MOD_RES (3)..(3): Xaa is D-Arg
  MOD_RES (4)..(4): Xaa is D-Arg
  MOD_RES (5)..(5): Xaa is D-Arg
  MOD_RES (6)..(6): Xaa is D-Ala
  MOD_RES (7)..(7): Xaa is D-Arg amidated
  BINDING (1)..(1): Xaa is Cys linked to Cys in SEQ ID NO: 3 via a disulfide bond
XXXXXXX

SEQ ID NO: 9 - protein, 7 aa, Artificial Sequence
  MOD_RES (1)..(1): Xaa is D-Cys acetylated
  MOD_RES (2)..(2): Xaa is D-Ala
  MOD_RES (3)..(3): Xaa is D-Arg
  MOD_RES (4)..(4): Xaa is D-Arg
  MOD_RES (5)..(5): Xaa is D-Arg
  MOD_RES (6)..(6): Xaa is D-Ala
  MOD_RES (7)..(7): Xaa is D-Arg amidated
  BINDING (1)..(1): Xaa is Cys linked to Cys in SEQ ID NO: 4 via a disulfide bond
XXXXXXX

SEQ ID NO: 10 - protein, 7 aa, Artificial Sequence
  MOD_RES (1)..(1): Xaa is D-Cys acetylated
  MOD_RES (2)..(2): Xaa is D-Ala
  MOD_RES (3)..(3): Xaa is D-Arg
  MOD_RES (4)..(4): Xaa is D-Arg
  MOD_RES (5)..(5): Xaa is D-Arg
  MOD_RES (6)..(6): Xaa is D-Ala
  MOD_RES (7)..(7): Xaa is D-Arg amidated
  BINDING (1)..(1): Xaa is Cys linked to Cys in SEQ ID NO: 5 via a disulfide bond
XXXXXXX

SEQ ID NO: 11 - protein, 7 aa, Artificial Sequence
  MOD_RES (1)..(1): Xaa is D-Cys acetylated
  MOD_RES (2)..(2): Xaa is D-Ala
  MOD_RES (3)..(3): Xaa is D-Arg
  MOD_RES (4)..(4): Xaa is D-Arg
  MOD_RES (5)..(5): Xaa is D-Arg
  MOD_RES (6)..(6): Xaa is D-Ala
  MOD_RES (7)..(7): Xaa is D-Arg amidated
  BINDING (1)..(1): Xaa is Cys linked to Cys in SEQ ID NO: 6 via a disulfide bond
XXXXXXX

SEQ ID NO: 12 - protein, 6 aa, Artificial Sequence
  MOD_RES (1)..(1): Xaa is D-Tyr
  MOD_RES (2)..(2): Xaa is D-His
  MOD_RES (3)..(3): Xaa is D-Tyr
XXXGGC

SEQ ID NO: 13 - protein, 6 aa, Artificial Sequence
  MOD_RES (1)..(1): Xaa is D-Tyr
  MOD_RES (2)..(2): Xaa is D-Pro
  MOD_RES (3)..(3): Xaa is D-Phe
XXXGGC

SEQ ID NO: 14 - protein, 6 aa, Artificial Sequence
  MOD_RES (1)..(1): Xaa is D-Tyr
  UNSURE (2)..(2): Xaa is Aib
  MOD_RES (3)..(3): Xaa is D-Phe
  MOD_RES (1)..(6): Cyclic peptide
XXXGGC

SEQ ID NO: 15 - protein, 6 aa, Artificial Sequence
  MOD_RES (1)..(1): Xaa is D-Tyr
  MOD_RES (2)..(2): Xaa is D-Arg
  MOD_RES (3)..(3): Xaa is D-Phe
  MOD_RES (1)..(6): Cyclic peptide
XXXGGC

SEQ ID NO: 16 - protein, 6 aa, Artificial Sequence
  MOD_RES (1)..(6): Cyclic peptide
YGFGGC

SEQ ID NO: 17 - protein, 6 aa, Artificial Sequence
  MOD_RES (1)..(1): Xaa is D-Tyr
  MOD_RES (3)..(3): Xaa is D-Phe
  MOD_RES (6)..(6): Xaa is D-Cys
  MOD_RES (1)..(6): Cyclic peptide
XGXGGX

SEQ ID NO: 18 - protein, 6 aa, Artificial Sequence
  MOD_RES (1)..(1): Xaa is D-Cys
  MOD_RES (4)..(4): Xaa is D-Phe
  MOD_RES (6)..(6): Xaa is D-Tyr
  MOD_RES (1)..(6): Cyclic peptide
XGGXGX

SEQ ID NO: 19 - protein, 7 aa, Artificial Sequence
  MOD_RES (1)..(1): Xaa is D-Cys acetylated
  MOD_RES (2)..(2): Xaa is D-Arg
  MOD_RES (3)..(3): Xaa is D-Lys
  MOD_RES (4)..(4): Xaa is D-Lys
  MOD_RES (5)..(5): Xaa is D-Arg
  MOD_RES (6)..(6): Xaa is D-Ala
  MOD_RES (7)..(7): Xaa is D-Arg amidated
  BINDING (1)..(1): Xaa is Cys linked to Cys in SEQ ID NO: 2 via a disulfide bond
XXXXXXX

SEQ ID NO: 20 - protein, 7 aa, Artificial Sequence
  MOD_RES (1)..(1): Xaa is D-Cys acetylated
  MOD_RES (2)..(2): Xaa is D-Arg
  MOD_RES (3)..(3): Xaa is D-Arg
  MOD_RES (4)..(4): Xaa is D-Ala
  MOD_RES (5)..(5): Xaa is D-Arg
  MOD_RES (6)..(6): Xaa is D-Ala
  MOD_RES (7)..(7): Xaa is D-Arg amidated
  BINDING (1)..(1): Xaa is Cys linked to Cys in SEQ ID NO: 5 via a disulfide bond
XXXXXXX

SEQ ID NO: 21 - protein, 7 aa, Artificial Sequence
  MOD_RES (1)..(1): Xaa is D-Cys acetylated
  MOD_RES (2)..(2): Xaa is D-Ala
  MOD_RES (3)..(3): Xaa is D-Arg
  MOD_RES (4)..(4): Xaa is D-Arg
  MOD_RES (5)..(5): Xaa is D-Arg
  MOD_RES (6)..(6): Xaa is D-Ala
  MOD_RES (7)..(7): Xaa is D-Arg amidated
  BINDING (1)..(1): Xaa is Cys linked to Cys in SEQ ID NO: 12 via a disulfide bond
XXXXXXX

SEQ ID NO: 22 - protein, 7 aa, Artificial Sequence
  MOD_RES (1)..(1): Xaa is D-Cys acetylated
  MOD_RES (2)..(2): Xaa is D-Ala
  MOD_RES (3)..(3): Xaa is D-Arg
  MOD_RES (4)..(4): Xaa is D-Arg
  MOD_RES (5)..(5): Xaa is D-Arg
  MOD_RES (6)..(6): Xaa is D-Ala
  MOD_RES (7)..(7): Xaa is D-Arg amidated
  BINDING (1)..(1): Xaa is Cys is linked to Cys in SEQ ID NO: 13 via a disulfide bond
XXXXXXX

SEQ ID NO: 23 - protein, 7 aa, Artificial Sequence
  MOD_RES (1)..(1): Xaa is D-Cys acetylated
  MOD_RES (2)..(2): Xaa is D-Ala
  MOD_RES (3)..(3): Xaa is D-Arg
  MOD_RES (4)..(4): Xaa is D-Arg
  MOD_RES (5)..(5): Xaa is D-Arg
  MOD_RES (6)..(6): Xaa is D-Ala
  MOD_RES (7)..(7): Xaa is D-Arg amidated
  BINDING (1)..(1): Xaa is Cys linked to Cys in SEQ ID NO: 14 via a disulfide bond
XXXXXXX

SEQ ID NO: 24 - protein, 7 aa, Artificial Sequence
  MOD_RES (1)..(1): Xaa is D-Cys acetylated
  MOD_RES (2)..(2): Xaa is D-Ala
  MOD_RES (3)..(3): Xaa is D-Arg
  MOD_RES (4)..(4): Xaa is D-Arg
  MOD_RES (5)..(5): Xaa is D-Arg
  MOD_RES (6)..(6): Xaa is D-Ala
  MOD_RES (7)..(7): Xaa is D-Arg amidated
  BINDING (1)..(1): Xaa is Cys linked to Cys in SEQ ID NO: 15 via a disulfide bond
XXXXXXX

SEQ ID NO: 25 - protein, 7 aa, Artificial Sequence
  MOD_RES (1)..(1): Xaa is D-Cys acetylated
  MOD_RES (2)..(2): Xaa is D-Ala
  MOD_RES (3)..(3): Xaa is D-Arg
  MOD_RES (4)..(4): Xaa is D-Arg
  MOD_RES (5)..(5): Xaa is D-Arg
  MOD_RES (6)..(6): Xaa is D-Ala
  MOD_RES (7)..(7): Xaa is D-Arg amidated
  BINDING (1)..(1): Xaa is Cys linked to Cys in SEQ ID NO: 16 via a disulfide bond
XXXXXXX

SEQ ID NO: 26 - protein, 7 aa, Artificial Sequence
  MOD_RES (1)..(1): Xaa is D-Cys acetylated
  MOD_RES (2)..(2): Xaa is D-Ala
  MOD_RES (3)..(3): Xaa is D-Arg
  MOD_RES (4)..(4): Xaa is D-Arg
  MOD_RES (5)..(5): Xaa is D-Arg
  MOD_RES (6)..(6): Xaa is D-Ala
  MOD_RES (7)..(7): Xaa is D-Arg amidated
  BINDING (1)..(1): Xaa is Cys linked to Cys in SEQ ID NO: 17 via a disulfide bond
XXXXXXX

SEQ ID NO: 27 - protein, 7 aa, Artificial Sequence
  MOD_RES (1)..(1): Xaa is D-Cys acetylated
  MOD_RES (2)..(2): Xaa is D-Ala
  MOD_RES (3)..(3): Xaa is D-Arg
  MOD_RES (4)..(4): Xaa is D-Arg
  MOD_RES (5)..(5): Xaa is D-Arg
  MOD_RES (6)..(6): Xaa is D-Ala
  MOD_RES (7)..(7): Xaa is D-Arg amidated
  BINDING (1)..(1): Xaa is Cys linked to Cys in SEQ ID NO: 18 via a disulfide bond
XXXXXXX

SEQ ID NO: 28 - protein, 7 aa, Artificial Sequence
  Linker
SGGSGGS